European Patent Application EP 4 644 547 A1, published November 5, 2025. Title: 5'-UTR VARIANT SEQUENCE AND USE THEREOF. Applicant: CJ CHEILJEDANG CORPORATION. Application KR. The sequence listing filed with the application follows.

SEQUENCE LISTING (17 sequences)

SEQ ID NO: 1 - DNA, 1143 bp, Corynebacterium glutamicum
  source 1..1143: mol_type = genomic DNA
  5'UTR 1..555
  misc_feature 556..558: note = start codon
gactaggtgagtgggcttaggtgtctcagagcacagtagtcggacattagagagctgcaccgcagtaaaaggccacgatgtaggaggtgggcggagtgtccgtgctgggaaactggcggggaacttttagagataaccctccgaattgctggcaaatttctgatgaaatttctccgcgaagcccacatgaactacccccgtttaccctcaaaataagccctgtgacacacataacaccccctaatcgtacccgctcacacgctattttcgaggtgtggttcgccttcggaaacgaatgcccccgccccacttggataaaagacgaattcacctgttagtctataacgcgggttgaaccgagaaacccctcaaggcagcagacaatagccgcaaggggttttgcggagcacgtcccctgtgatcgttgcgctgatgtgcgacggagtccgtagcgattacagcgagtttttcagacgtccatcgcaccgtgcacaacaacatttcaggtgcacggcccgaacacgggagagaacgctgagcgttacaacactgtccatgaagggcgaattccacgcccccgatttggacaaagaatttttcccggggcacgtaaccgatagtggtgaagtcgtgaacatgctgttcaccgatttcgctaatggttggttcgcaatggaccgcatcgtattgatccgtcttcttatgacggcagtcgttgtggtcttcttcctttgggctatgcgcaagccaaagcttgttccgcatggcgtccagaattttgcagagtacgcactcgatttcgttcgtattcacatcgctgaagacatcctcggaaagaaggaaggtcgtcggttcctgccgatcctggccaccatcttcttcgcggctctgttgatgaaccttgcaacgatcatcccgggactaaacatctcctccaactcacgtattgcattcccaatcgtgatggcggtagctggttacatcgcgtttatctacgcaggctctaagcgttacggattcttcaaatatgtgaagtcttctgttgtgattccgaacattccaccagcacttcacgtcttggtggttccaattgagttcttctctacattcatcttgaggccagtcaccctggcactgcgtttg

SEQ ID NO: 2 - DNA, 40 bp, synthetic construct
  source 1..40: mol_type = other DNA
agaacgctgagtcggacaacactgtccatgaagggcgaat

SEQ ID NO: 3 - DNA, 40 bp, synthetic construct
  source 1..40: mol_type = other DNA
ctctagaggatcccccaaacgcagtgccagggtgactggc

SEQ ID NO: 4 - DNA, 40 bp, synthetic construct
  source 1..40: mol_type = other DNA
gacagtgttgtactccttagcgttctctcccgtgttcggg

SEQ ID NO: 5 - DNA, 40 bp, synthetic construct
  source 1..40: mol_type = other DNA
agaacgctaaggagtacaacactgtccatgaagggcgaat

SEQ ID NO: 6 - DNA, 40 bp, synthetic construct
  source 1..40: mol_type = other DNA
tgttgtcctcctcagcgttctctcccgtgttcgggccgtg

SEQ ID NO: 7 - DNA, 40 bp, synthetic construct
  source 1..40: mol_type = other DNA
gagaacgctgaggaggacaacactgtccatgaagggcgaa

SEQ ID NO: 8 - DNA, 40 bp, synthetic construct
  source 1..40: mol_type = other DNA
agtgttggcctcctcagcgttctctcccgtgttcgggccg

SEQ ID NO: 9 - DNA, 40 bp, synthetic construct
  source 1..40: mol_type = other DNA
agagaacgctgaggaggccaacactgtccatgaagggcga

SEQ ID NO: 10 - DNA, 20 bp, synthetic construct
  source 1..20: mol_type = other DNA
atcgccattcgccattcagg

SEQ ID NO: 11 - DNA, 20 bp, synthetic construct
  source 1..20: mol_type = other DNA
tcattaatgcagctggcacg

SEQ ID NO: 12 - DNA, 60 bp, Corynebacterium glutamicum
  source 1..60: mol_type = genomic DNA; note = atpB wild type
aacgctgagcgttacaacactgtccatgaagggcgaattccacgcccccgatttggacaa

SEQ ID NO: 13 - DNA, 25 bp, Corynebacterium glutamicum
  source 1..25: mol_type = genomic DNA; note = wild type RBS
aacgctgagcgttacaacactgtcc

SEQ ID NO: 14 - DNA, 25 bp, synthetic construct
  source 1..25: mol_type = other DNA; note = RBS 1
aacgctgagtcggacaacactgtcc

SEQ ID NO: 15 - DNA, 25 bp, synthetic construct
  source 1..25: mol_type = other DNA; note = RBS 2
aacgctgaggaggacaacactgtcc

SEQ ID NO: 16 - DNA, 25 bp, synthetic construct
  source 1..25: mol_type = other DNA; note = RBS 3
aacgctgaggaggccaacactgtcc

SEQ ID NO: 17 - DNA, 35 bp, Corynebacterium glutamicum
  source 1..35: mol_type = genomic DNA; note = protein coding sequence
atgaagggcgaattccacgcccccgatttggacaa